European Patent Specification EP 3 405 496 B1, published October 25, 2023. Title: ROR1 Antibody Compositions and Related Methods. Applicant: NBE-Therapeutics AG The Scripps Research Institute. The sequence listing filed with the application follows.

SEQUENCE LISTING (161 sequences)

SEQ ID NO: 1 - protein, 117 aa, Oryctolagus cuniculus
QEQQKESGGGLFKPTDTLTLTCTASGFDISSYYMSWVRQAPGNGLEWIGAIGISGNAYYASWAKSRSTITRNTNLNTVTLKMTSLTAADTATYFCARDHPTYGMDLWGPGTLVTVSS

SEQ ID NO: 2 - protein, 118 aa, Oryctolagus cuniculus
QEQLEESGGGLVTPGGSLTLTCTASGFTISTYHMSWVRQAPGKGLEWIGSIYAGSGSTYYASWVNGRFTISSNTTQNTVSLQMNSLTVADTATYFCARDHPSYGMDLWGPGTLVTVSS

SEQ ID NO: 3 - protein, 125 aa, Oryctolagus cuniculus
QEQLKESGGGLVQPGGSLKLSCKASGFDLSNYGVSWVRQAPGKGLEWIGYIDPTFDYTYYASWVNGRFSISRENTQNTVSLQINSLTPADTATYFCARWVYGVDDYGDGNWLDLWGQGTLVTISS

SEQ ID NO: 4 - protein, 117 aa, Oryctolagus cuniculus
QEQLEESGGRLVTPGTPLTLTCTASGFFLSSYYVSWVRQAPGKGLEWIGAIGTGGSAYYASWAKSRSTITRNTNLSTVTLKMTSLTAADTATYFCARDHPNYGMDLWGPGTLVTVSS

SEQ ID NO: 5 - protein, 113 aa, Oryctolagus cuniculus
QSLEESGGGLVQPGESLTLTCTVSGFSLSRNGMTWVRQAPGKGLEWIGIITSSGDKYYATWAKGRFTISKTSSTTVDLKMTSLTTEDTATYFCARGTVSSDIWGPGTLVTISS

SEQ ID NO: 6 - protein, 115 aa, Oryctolagus cuniculus
QEQLKESGRGLVQPGGSLKLSCKASGFDFSGWYMTWVRQAPGKGLEWIGTIGTTKGRTYYASWVNGRFTISSNAQNTVDLQMNSLTAADRATYFCVRGSDYFDLWGPGTLVTISS

SEQ ID NO: 7 - protein, 120 aa, Oryctolagus cuniculus
QEQLVESGGRLVTPGGSLTLTCTASGFSLSSYYMGWVRQAPGKGLEWIGTIYGGSGSTWYASWVKGRFTISKTSTAVDLKITSLTTEDTATYFCARSYPGWTTEPYFDIWGPGTLVTVSS

SEQ ID NO: 8 - protein, 121 aa, Oryctolagus cuniculus
QSVEESGGRLVTPGTPLTLTCTASGIDLSRYAVNWVRQAPGKGLEWIGVISGSGTTYYASWAKGRFTISKTSTTVDLKITSPTTEDTATYFCARGWATDGIFDYDDTFNLWGPGTLVTVSS

SEQ ID NO: 9 - protein, 115 aa, Oryctolagus cuniculus
QEQLVESGGRLVTPGGSLTLTCAASGFSPSSYWMSWVRQAPGKGLEWIGAIYVDSGSAYYASWAKSRFTISKTSSTTVDLKMTSLTTEDTAIYFCARDGWGSDVWGPGTLVTISS

SEQ ID NO: 10 - protein, 113 aa, Oryctolagus cuniculus
QSLEESGGRLVTPGTPLTLTCTVSGFSLSSYYMSWVRQAPGKGLEWIGTISSSGSTYYASWVKGRFTISKTSTTVDLKMTSLTTEDTATYFCARDLDYDMDLWGPGTLVTVSS

SEQ ID NO: 11 - protein, 117 aa, Oryctolagus cuniculus
QEQLEESGGRLVTPGTPLTLTCTASGFSLSNYYMSWVRQAPGKGLEYIGIISSSGSTYYASWAKGRFTISKTSSTTVDLKITSPTTEDTATYFCARLYVSDSTANLWGPGTLVTVSS

SEQ ID NO: 12 - protein, 114 aa, Oryctolagus cuniculus
QSLEESGGRLVTPGTPLTLTCTVSGFSLSSYWMSWVRQAPGKGLEWIGAIYGSGNTYYASWAKGRFTISKTSTTVDLKITSPTTEDTATYFCARDVHSTATDLWGPGTLVTISS

SEQ ID NO: 13 - protein, 115 aa, Oryctolagus cuniculus
QSLEESGGRLVTPGTPLTLTCTASGFSLSDYYMSWVRQAPGEGLEWIGTIYGGSGNTWYATWAKGRFTISKTSTTVDLKITSPTTEDTATYFCARDFGLSTGGLWGPGTLVTISS

SEQ ID NO: 14 - protein, 107 aa, Oryctolagus cuniculus
SYELTQLPSVSVSLGQTARITCEGNNIGSKAVHWYQQKPGLAPGLLIYDDDERPSGVPDRFSGSNSGDTATLTISGAQAGDEADYYCQVWDSSAYVFGGGTQLTVTG

SEQ ID NO: 15 - protein, 109 aa, Oryctolagus cuniculus
SYELTQLPSVSVSLGQTARITCGGNSIGSKAVNWYQQKPGLAPGLLIYDDDERPSGVPDRFSASNSGDTATLTISGAQAEDEADYYCQLWDSSAVAYVFGGGTQLTVTG

SEQ ID NO: 16 - protein, 112 aa, Oryctolagus cuniculus
QFVLTQSPSVSAALGASAKLTCTLSSAHKTYTIDWYQQQQGEAPRYLMELKSDGSYTKGTGVPDRFSGSSSGADRYLIIPSVQADDEADYYCGTDYSGGYVFGGGTQLTVTG

SEQ ID NO: 17 - protein, 109 aa, Oryctolagus cuniculus
SYELTQLPSVSVSLGQTARITCGGNSIGSKAVNWYQQKPGLAPGLLIYDDDERPSGVPDRFSGSNSGDTATLTISGAQAGDEADYYCQLWDSSTGAYAFGGGTQLTVTG

SEQ ID NO: 18 - protein, 112 aa, Oryctolagus cuniculus
ELVLTQTPSPVSAAVGGTVTINCQASQSVYGNNELAWYQQKPGQPPKLLIYRASILTSGVPSRFKGSGSGTQFTLTISNVQREDAATYYCLGGYVSQSYRAAFGGGTELEIL

SEQ ID NO: 19 - protein, 109 aa, Oryctolagus cuniculus
SYELTQLPSVSVSLGQTARITCGGNSIGSKAVNWYQQKPGLAPGLLIYDDDERPSGVPARFSGSNSGDTATLTISGAQAGDEADYYCQLWDSSAGAYVFGGGTQLTVTG

SEQ ID NO: 20 - protein, 111 aa, Oryctolagus cuniculus
QFVLTQPQSVSGSLGQTVSISCNRDSGNIEDYYVHWYQQHPGKAPTTVIYNDDQRPSGVPDRFSGSIDSTSNSASLTITGLLAEDEADYYCLSSDSSAYVFGGGTQLTVTG

SEQ ID NO: 21 - protein, 107 aa, Oryctolagus cuniculus
SYELTQLPSVSVSLGQTARITCGGDSIESKAVHWYQQKPGLAPGLLVYNDDERPSGVPDRFSGSNSGDTATLTISGAQAGDEADYYCQLWDGSAYVFGGGTQLTVTG

SEQ ID NO: 22 - protein, 109 aa, Oryctolagus cuniculus
SYELTQLPSVSVSLGQTARITCGGNSIGSKAVHWYQQKPGLAPGLLIYDDDERPSGVPDRFSGSNSGDTATLTISGAQAGDEADYYCQLWDSSAGAYVFGGGTQLTVTG

SEQ ID NO: 23 - protein, 107 aa, Oryctolagus cuniculus
SYELTQLPSVSVSLGQTARITCGGNSIGSKAVHWYQQKPGLAPGLLIYNDDERPSGVPDRFSGSNSGDTATLTISGAQAGDEADYYCQLWDNNAAVFGGGTQLTVTG

SEQ ID NO: 24 - protein, 110 aa, Oryctolagus cuniculus
DIVLTQTPSSTSAAVGGTVTIKCQASQSIDSYLAWYQQKPGQPPKLLIYGASNLASGVPSRFSGSRSGTEYILTISGVQREDAATYYCLGGYPNYFHRTAFGGGTKLEIK

SEQ ID NO: 25 - protein, 109 aa, Oryctolagus cuniculus
SYELTQLPSVSVSLGQTARITCGGNNIGSKAVNWYQQKPGLAPGLLIYNDDERPSGVPDRFSGSNSGDTATLTISGAQAGDEADYYCQLWDSSAGAYVFGGGTQLTVTG

SEQ ID NO: 26 - protein, 109 aa, Oryctolagus cuniculus
SYELTQLPSVSVSLGQTARITCGGNSIGSKAVNWYQQKPGLAPGLLIYDDDERPSGVPDRFSGSNSGDTATLTISGAQAGDEADYYCQLWDSSARAFVFGGGTQLTVTG

SEQ ID NO: 27 - protein, 5 aa, Oryctolagus cuniculus
SYYMS

SEQ ID NO: 28 - protein, 16 aa, Oryctolagus cuniculus
AIGISGNAYYASWAKS

SEQ ID NO: 29 - protein, 9 aa, Oryctolagus cuniculus
DHPTYGMDL

SEQ ID NO: 30 - protein, 5 aa, Oryctolagus cuniculus
TYHMS

SEQ ID NO: 31 - protein, 17 aa, Oryctolagus cuniculus
SIYAGSGSTYYASWVNG

SEQ ID NO: 32 - protein, 9 aa, Oryctolagus cuniculus
DHPSYGMDL

SEQ ID NO: 33 - protein, 5 aa, Oryctolagus cuniculus
NYGVS

SEQ ID NO: 34 - protein, 17 aa, Oryctolagus cuniculus
YIDPTFDYTYYASWVNG

SEQ ID NO: 35 - protein, 16 aa, Oryctolagus cuniculus
WVYGVDDYGDGNWLDL

SEQ ID NO: 36 - protein, 5 aa, Oryctolagus cuniculus
SYYVS

SEQ ID NO: 37 - protein, 16 aa, Oryctolagus cuniculus
AIGTGGSAYYASWAKS

SEQ ID NO: 38 - protein, 9 aa, Oryctolagus cuniculus
DHPNYGMDL

SEQ ID NO: 39 - protein, 5 aa, Oryctolagus cuniculus
RNGMT

SEQ ID NO: 40 - protein, 16 aa, Oryctolagus cuniculus
IITSSGDKYYATWAKG

SEQ ID NO: 41 - protein, 7 aa, Oryctolagus cuniculus
GTVSSDI

SEQ ID NO: 42 - protein, 5 aa, Oryctolagus cuniculus
GWYMT

SEQ ID NO: 43 - protein, 17 aa, Oryctolagus cuniculus
TIGTTKGRTYYASWVNG

SEQ ID NO: 44 - protein, 7 aa, Oryctolagus cuniculus
GSDYFDL

SEQ ID NO: 45 - protein, 5 aa, Oryctolagus cuniculus
SYYMG

SEQ ID NO: 46 - protein, 17 aa, Oryctolagus cuniculus
TIYGGSGSTWYASWVKG

SEQ ID NO: 47 - protein, 13 aa, Oryctolagus cuniculus
SYPGWTTEPYFDI

SEQ ID NO: 48 - protein, 5 aa, Oryctolagus cuniculus
RYAVN

SEQ ID NO: 49 - protein, 16 aa, Oryctolagus cuniculus
VISGSGTTYYASWAKG

SEQ ID NO: 50 - protein, 16 aa, Oryctolagus cuniculus
GWATDGIFDYDDTFNL

SEQ ID NO: 51 - protein, 5 aa, Oryctolagus cuniculus
SYWMS

SEQ ID NO: 52 - protein, 17 aa, Oryctolagus cuniculus
AIYVDSGSAYYASWAKS

SEQ ID NO: 53 - protein, 7 aa, Oryctolagus cuniculus
DGWGSDV

SEQ ID NO: 54 - protein, 5 aa, Oryctolagus cuniculus
SYYMS

SEQ ID NO: 55 - protein, 16 aa, Oryctolagus cuniculus
TISSSGSTYYASWVKG

SEQ ID NO: 56 - protein, 10 aa, Oryctolagus cuniculus
LYVSDSTANL

SEQ ID NO: 57 - protein, 5 aa, Oryctolagus cuniculus
NYYMS

SEQ ID NO: 58 - protein, 16 aa, Oryctolagus cuniculus
IISSSGSTYYASWAKG

SEQ ID NO: 59 - protein, 10 aa, Oryctolagus cuniculus
LYVSDSTANL

SEQ ID NO: 60 - protein, 5 aa, Oryctolagus cuniculus
SYWMS

SEQ ID NO: 61 - protein, 16 aa, Oryctolagus cuniculus
AIYGSGNTYYASWAKG

SEQ ID NO: 62 - protein, 9 aa, Oryctolagus cuniculus
DVHSTATDL

SEQ ID NO: 63 - protein, 5 aa, Oryctolagus cuniculus
DYYMS

SEQ ID NO: 64 - protein, 17 aa, Oryctolagus cuniculus
TIYGGSGNTWYATWAKG

SEQ ID NO: 65 - protein, 9 aa, Oryctolagus cuniculus
DFGLSTGGL

SEQ ID NO: 66 - protein, 11 aa, Oryctolagus cuniculus
EGNNIGSKAVH

SEQ ID NO: 67 - protein, 7 aa, Oryctolagus cuniculus
DDDERPS

SEQ ID NO: 68 - protein, 9 aa, Oryctolagus cuniculus
QVWDSSAYV

SEQ ID NO: 69 - protein, 11 aa, Oryctolagus cuniculus
GGNSIGSKAVN

SEQ ID NO: 70 - protein, 7 aa, Oryctolagus cuniculus
DDDERPS

SEQ ID NO: 71 - protein, 11 aa, Oryctolagus cuniculus
QLWDSSAVAYV

SEQ ID NO: 72 - protein, 12 aa, Oryctolagus cuniculus
TLSSAHKTYTID

SEQ ID NO: 73 - protein, 11 aa, Oryctolagus cuniculus
LKSDGSYTKGT

SEQ ID NO: 74 - protein, 9 aa, Oryctolagus cuniculus
GTDYSGGYV

SEQ ID NO: 75 - protein, 11 aa, Oryctolagus cuniculus
GGNSIGSKAVN

SEQ ID NO: 76 - protein, 7 aa, Oryctolagus cuniculus
DDDERPS

SEQ ID NO: 77 - protein, 11 aa, Oryctolagus cuniculus
QLWDSSTGAYA

SEQ ID NO: 78 - protein, 13 aa, Oryctolagus cuniculus
QASQSVYGNNELA

SEQ ID NO: 79 - protein, 7 aa, Oryctolagus cuniculus
RASILTS

SEQ ID NO: 80 - protein, 12 aa, Oryctolagus cuniculus
LGGYVSQSYRAA

SEQ ID NO: 81 - protein, 11 aa, Oryctolagus cuniculus
GGNSIGSKAVN

SEQ ID NO: 82 - protein, 7 aa, Oryctolagus cuniculus
DDDERPS

SEQ ID NO: 83 - protein, 11 aa, Oryctolagus cuniculus
QLWDSSAGAYV

SEQ ID NO: 84 - protein, 13 aa, Oryctolagus cuniculus
NRDSGNIEDYYVH

SEQ ID NO: 85 - protein, 7 aa, Oryctolagus cuniculus
NDDQRPS

SEQ ID NO: 86 - protein, 9 aa, Oryctolagus cuniculus
LSSDSSAYV

SEQ ID NO: 87 - protein, 11 aa, Oryctolagus cuniculus
GGDSIESKAVH

SEQ ID NO: 88 - protein, 7 aa, Oryctolagus cuniculus
NDDERPS

SEQ ID NO: 89 - protein, 9 aa, Oryctolagus cuniculus
QLWDGSAYV

SEQ ID NO: 90 - protein, 11 aa, Oryctolagus cuniculus
GGNSIGSKAVH

SEQ ID NO: 91 - protein, 7 aa, Oryctolagus cuniculus
DDDERPS

SEQ ID NO: 92 - protein, 11 aa, Oryctolagus cuniculus
QLWDSSAGAYV

SEQ ID NO: 93 - protein, 11 aa, Oryctolagus cuniculus
GGNSIGSKAVH

SEQ ID NO: 94 - protein, 7 aa, Oryctolagus cuniculus
NDDERPS

SEQ ID NO: 95 - protein, 9 aa, Oryctolagus cuniculus
QLWDNNAAV

SEQ ID NO: 96 - protein, 11 aa, Oryctolagus cuniculus
QASQSIDSYLA

SEQ ID NO: 97 - protein, 7 aa, Oryctolagus cuniculus
GASNLAS

SEQ ID NO: 98 - protein, 12 aa, Oryctolagus cuniculus
LGGYPNYFHRTA

SEQ ID NO: 99 - protein, 11 aa, Oryctolagus cuniculus
GGNNIGSKAVN

SEQ ID NO: 100 - protein, 7 aa, Oryctolagus cuniculus
NDDERPS

SEQ ID NO: 101 - protein, 11 aa, Oryctolagus cuniculus
QLWDSSAGAYV

SEQ ID NO: 102 - protein, 11 aa, Oryctolagus cuniculus
GGNSIGSKAVN

SEQ ID NO: 103 - protein, 7 aa, Oryctolagus cuniculus
DDDERPS

SEQ ID NO: 104 - protein, 11 aa, Oryctolagus cuniculus
QLWDSSARAFV

SEQ ID NO: 105 - DNA, 60 bp, Artificial sequence
  Synthetic sequence
atcctgtttctcgtagctgctgcaactggagcacactccgcccggggcgccgccgcccag

SEQ ID NO: 106 - DNA, 60 bp, Artificial sequence
  Synthetic sequence
ccactcgatcttctgggcctcgaagatgtcgttcaggccctccatcttgttcttctcctt

SEQ ID NO: 107 - DNA, 60 bp, Artificial sequence
  Synthetic sequence
gctgggtaccggcgcgccaccatggactggacttggagaatcctgtttctcgtagctgct

SEQ ID NO: 108 - DNA, 60 bp, Artificial sequence
  Synthetic sequence
gccggcctcgagtcagtgatggtgatggtggtgctcgtgccactcgatcttctgggcctc

SEQ ID NO: 109 - DNA, 99 bp, Artificial sequence
  Synthetic sequence
gctgggtaccggcgcgccaccatggactggacttggagaatcctgtttctcgtagctgctgcaactggagcacactccgcccggggcgccgccgcccag

SEQ ID NO: 110 - DNA, 52 bp, Artificial sequence
  Synthetic sequence
cggcctcgagtcagtgatggtgatggtggtgctccatcttgttcttctcctt

SEQ ID NO: 111 - DNA, 99 bp, Artificial sequence
  Synthetic sequence
gctgggtaccggcgcgccaccatggactggacttggagaatcctgtttctcgtagctgctgcaactggagcacactccgaagtggaggttctggatccg

SEQ ID NO: 112 - DNA, 52 bp, Artificial sequence
  Synthetic sequence
cggcctcgagtcagtgatggtgatggtggtgccccatcttgctgctgtctcg

SEQ ID NO: 113 - DNA, 41 bp, Artificial sequence
  Synthetic sequence
gaggaggagctcactctcaggagcagcagaaggagtccggg

SEQ ID NO: 114 - DNA, 60 bp, Artificial sequence
  Synthetic sequence
cgatgggcccttggtggaggctgaagagacggtgacgagggtccctggcccccagaggtc

SEQ ID NO: 115 - DNA, 60 bp, Artificial sequence
  Synthetic sequence
gagaagcttgttgctctggatctctggtgcctacgggtcctatgagctgacacagctgcc

SEQ ID NO: 116 - DNA, 21 bp, Artificial sequence
  Synthetic sequence
ggccatggctggttgggcagc

SEQ ID NO: 117 - DNA, 60 bp, Artificial sequence
  Synthetic sequence
ggtaccggcgcgccaccatggactggacttggagaatcctgtttctcgtagctgctgcaa

SEQ ID NO: 118 - DNA, 20 bp, Artificial sequence
  Synthetic sequence
gccgctggtcagggctcctg

SEQ ID NO: 119 - DNA, 20 bp, Artificial sequence
  Synthetic sequence
caggagccctgaccagcggc

SEQ ID NO: 120 - DNA, 30 bp, Artificial sequence
  Synthetic sequence
ggcctcgagtcatttacccggagacaggga

SEQ ID NO: 121 - DNA, 54 bp, Artificial sequence
  Synthetic sequence
tttctcgtagctgctgcaactggagcacactcccagtcgctggaggagtccggg

SEQ ID NO: 122 - protein, 54 aa, Artificial sequence
  Synthetic sequence
TTTCTCGTAGCTGCTGCAACTGGAGCACACTCCCAGTCGTTGGAGGAGTCCGGG

SEQ ID NO: 123 - DNA, 54 bp, Artificial sequence
  Synthetic sequence
tttctcgtagctgctgcaactggagcacactcccagtcgttggaggagtccggg

SEQ ID NO: 124 - protein, 36 aa, Artificial sequence
  Synthetic sequence
GGAGGGCGCCAGGGGGAAGACCGATGGGCCCTTGGT

SEQ ID NO: 125 - DNA, 54 bp, Artificial sequence
  Synthetic sequence
tttctcgtagctgctgcaactggagcacactcctcctatgagctgacacagctg

SEQ ID NO: 126 - DNA, 54 bp, Artificial sequencee; identical to SEQ ID NO: 125
  Synthetic sequence

SEQ ID NO: 127 - DNA, 54 bp, Artificial sequence
  Synthetic sequence
tttctcgtagctgctgcaactggagcacactccgagctcgtgctgacccagact

SEQ ID NO: 128 - DNA, 30 bp, Artificial sequence
  Synthetic sequence
ggcctcgagttatgaacattctgtaggggc

SEQ ID NO: 129 - DNA, 30 bp, Artificial sequence
  Synthetic sequence
ggcctcgagttaacactctcccctgttgaa

SEQ ID NO: 130 - protein, 117 aa, Artificial sequence
  Synthetic sequence
QVQLRESGPGLVKPSETLSLTCTVSGFDISSYYMSWVRQPPGKGLEWIGAIGISGNAYYASWAKSRVTISRDTSKNQFSLKLSSVTAADTAVYYCARDHPTYGMDLWGPGTLVTVSS

SEQ ID NO: 131 - protein, 117 aa, Artificial sequence
  Synthetic sequence
QVQLQESGPGLVKPSETLSLTCTVSGFDISSYYMSWVRQPPGKGLEWIGAIGISGNAYYASWAKSRVTISRDTSKNQFSLKLSSVTAADTAVYYCARDHPTYGMDLWGPGTLVTVSS

SEQ ID NO: 132 - protein, 117 aa, Artificial sequence; identical to SEQ ID NO: 131
  Synthetic sequence

SEQ ID NO: 133 - protein, 117 aa, Artificial sequence; identical to SEQ ID NO: 130
  Synthetic sequence

SEQ ID NO: 134 - protein, 117 aa, Artificial sequence
  Synthetic sequence
QVQLQESGPGLVKPSETLSLTCTVSGFDISSYYMSWVRQPPGNGLEWIGAIGISGNAYYASWAKSRVTISRDTSKNQFSLKLSSVTAADTAVYYCARDHPTYGMDLWGPGTLVTVSS

SEQ ID NO: 135 - protein, 117 aa, Artificial sequence; identical to SEQ ID NO: 134
  Synthetic sequence

SEQ ID NO: 136 - protein, 107 aa, Artificial sequence
  Synthetic sequence
SYELTQPLSVSVALGQTARITCEGNNIGSKAVHWYQQKPGQAPVLVIYDDDERPSGIPERFSGSNSGNTATLTISRAQAGDEADYYCQVWDSSAYVFGGGTKLTVLG

SEQ ID NO: 137 - protein, 107 aa, Artificial sequence
  Synthetic sequence
SYELTQPPSVSVSPGQTAIITCEGNNIGSKAVHWYQQKPGLSPVLVIYDDDERPSGIPERFSGSNSGNTATLTVSGTQDMDEADYYCQVWDSSAYVFGGGTKLTVLG

SEQ ID NO: 138 - protein, 107 aa, Artificial sequence
  Synthetic sequence
SYELTQPPSVSVAPGKTARITCEGNNIGSKAVHWYQQKPGQAPVLVIYDDDERPSGIPERFSGSNSGNTATLTISRVEAGDEADYYCQVWDSSAYVFGGGTKLTVLG

SEQ ID NO: 139 - protein, 107 aa, Artificial sequence; identical to SEQ ID NO: 138
  Synthetic sequence

SEQ ID NO: 140 - protein, 107 aa, Artificial sequence; identical to SEQ ID NO: 138
  Synthetic sequence

SEQ ID NO: 141 - protein, 107 aa, Artificial sequence
  Synthetic sequence
SYELTQPLSVSVALGQTARITCEGNNIGSKAVHWYQQKPGLAPVLVIYDDDERPSGIPERFSGSNSGNTATLTISRAQAGDEADYYCQVWDSSAYVFGGGTQLTVLG

SEQ ID NO: 142 - protein, 5 aa, Artificial sequence
  Synthetic sequence
  MISC_FEATURE (3)..(3): X is any amino acid residue
LPXSG

SEQ ID NO: 143 - protein, 5 aa, Artificial sequence
  Synthetic sequence
  MISC_FEATURE (3)..(3): X is any amino acid residue
LPXAG

SEQ ID NO: 144 - protein, 5 aa, Artificial sequence
  Synthetic sequence
  MISC_FEATURE (3)..(3): X is any amino acid residue
LPXTG

SEQ ID NO: 145 - protein, 5 aa, Artificial sequence
  Synthetic sequence
  MISC_FEATURE (3)..(3): X is any amino acid residue
LAXTG

SEQ ID NO: 146 - protein, 5 aa, Artificial sequence
  Synthetic sequence
NPQTG

SEQ ID NO: 147 - protein, 4 aa, Artificial sequence
  Synthetic sequence
  MISC_FEATURE (3)..(3): X is any amino acid residue
LPXT

SEQ ID NO: 148 - protein, 460 aa, Artificial sequence
  Synthetic sequence
EIQLQQSGPVLVKPGASVKVSCKASGYAFTAYNIHWVRQSHGKRLEWIGSFDPYDGGSSYNQKFKDKATLTVDKSSTTAYMHLNSLTSEDSAVYYCARGWYYFDYWGHGTTLTVSSASTKGPSVFPLAPSSKSTSGGTAALGCLVKDYFPEPVTVSWNSGALTSGVHTFPAVLQSSGLYSLSSVVTVPSSSLGTQTYICNVNHKPSNTKVDKKVEPKSCDKTHTCPPCPAPELLGGPSVFLFPPKPKDTLMISRTPEVTCVVVDVSHEDPEVKFNWYVDGVEVHNAKTKPREEQYNSTYRVVSVLTVLHQDWLNGKEYKCKVSNKALPAPIEKTISKAKGQPREPQVYTLPPSRDELTKNQVSLTCLVKGFYPSDIAVEWESNGQPENNYKTTPPVLDSDGSFFLYSKLTVDKSRWQQGNVFSCSVMHEALHNHYTQKSLSLSPGKLPETGGWSHPQFEK

SEQ ID NO: 149 - protein, 233 aa, Artificial sequence
  Synthetic sequence
DVQITQSPSYLAASPGETITINCRASKSISKYLAWYQEKPGKTNKLLIYSGSTLQSGIPSRFRGSGSGTDFTLTISSLEPEDFAMYYCQQHDESPYTFGEGTKLEIKRTVAAPSVFIFPPSDEQLKSGTASVVCLLNNFYPREAKVQWKVDNALQSGNSQESVTEQDSKDSTYSLSSTLTLSKADYEKHKVYACEVTHQGLSSPVTKSFNRGECGGGGSLPETGGWSHPQFEK

SEQ ID NO: 150 - protein, 462 aa, Artificial sequence
  Synthetic sequence
QVQLQQSGAELVRPGASVTLSCKASGYTFSDYEMHWVIQTPVHGLEWIGAIDPETGGTAYNQKFKGKAILTADKSSSTAYMELRSLTSEDSAVYYCTGYYDYDSFTYWGQGTLVTVSAASTKGPSVFPLAPSSKSTSGGTAALGCLVKDYFPEPVTVSWNSGALTSGVHTFPAVLQSSGLYSLSSVVTVPSSSLGTQTYICNVNHKPSNTKVDKKVEPKSCDKTHTCPPCPAPELLGGPSVFLFPPKPKDTLMISRTPEVTCVVVDVSHEDPEVKFNWYVDGVEVHNAKTKPREEQYNSTYRVVSVLTVLHQDWLNGKEYKCKVSNKALPAPIEKTISKAKGQPREPQVYTLPPSRDELTKNQVSLTCLVKGFYPSDIAVEWESNGQPENNYKTTPPVLDSDGSFFLYSKLTVDKSRWQQGNVFSCSVMHEALHNHYTQKSLSLSPGKLPETGGWSHPQFEK

SEQ ID NO: 151 - protein, 233 aa, Artificial sequence
  Synthetic sequence
DIVMTQSQKIMSTTVGDRVSITCKASQNVDAAVAWYQQKPGQSPKLLIYSASNRYTGVPDRFTGSGSGTDFTLTISNMQSEDLADYFCQQYDIYPYTFGGGTKLEIKRTVAAPSVFIFPPSDEQLKSGTASVVCLLNNFYPREAKVQWKVDNALQSGNSQESVTEQDSKDSTYSLSSTLTLSKADYEKHKVYACEVTHQGLSSPVTKSFNRGECGGGGSLPETGGWSHPQFEK

SEQ ID NO: 152 - protein, 462 aa, Artificial sequence
  Synthetic sequence
EVQLVQSGAEVKKPGASVKVSCKASGYTFSDYEMHWVRQAPGQGLEWLGAIDPETGGTAYNQKFKGRVTMTGDTSISTAYMELSRLTSDDTAVYYCTGYYDYDSFTYWGQGTLVSVSSASTKGPSVFPLAPSSKSTSGGTAALGCLVKDYFPEPVTVSWNSGALTSGVHTFPAVLQSSGLYSLSSVVTVPSSSLGTQTYICNVNHKPSNTKVDKKVEPKSCDKTHTCPPCPAPELLGGPSVFLFPPKPKDTLMISRTPEVTCVVVDVSHEDPEVKFNWYVDGVEVHNAKTKPREEQYNSTYRVVSVLTVLHQDWLNGKEYKCKVSNKALPAPIEKTISKAKGQPREPQVYTLPPSRDELTKNQVSLTCLVKGFYPSDIAVEWESNGQPENNYKTTPPVLDSDGSFFLYSKLTVDKSRWQQGNVFSCSVMHEALHNHYTQKSLSLSPGKLPETGGWSHPQFEK

SEQ ID NO: 153 - protein, 233 aa, Artificial sequence
  Synthetic sequence
DIQMTQSPSSLSTSVGDRVTITCKASQNVDAAVAWYQQKPGKAPKLLIYSASNRYTGVASRFSGSGSGTDFTFTISSLQSEDLADYFCQQYDIYPYTFGQGTKLEIKRTVAAPSVFIFPPSDEQLKSGTASVVCLLNNFYPREAKVQWKVDNALQSGNSQESVTEQDSKDSTYSLSSTLTLSKADYEKHKVYACEVTHQGLSSPVTKSFNRGECGGGGSLPETGGWSHPQFEK

SEQ ID NO: 154 - protein, 460 aa, Artificial sequence
  Synthetic sequence
QSVKESEGDLVTPAGNLTLTCTASGSDINDYPISWVRQAPGKGLEWIGFINSGGSTWYASWVKGRFTISRTSTTVDLKMTSLTTDDTATYFCARGYSTYYGDFNIWGPGTLVTISSASTKGPSVFPLAPSSKSTSGGTAALGCLVKDYFPEPVTVSWNSGALTSGVHTFPAVLQSSGLYSLSSVVTVPSSSLGTQTYICNVNHKPSNTKVDKKVEPKSCDKTHTCPPCPAPELLGGPSVFLFPPKPKDTLMISRTPEVTCVVVDVSHEDPEVKFNWYVDGVEVHNAKTKPREEQYNSTYRVVSVLTVLHQDWLNGKEYKCKVSNKALPAPIEKTISKAKGQPREPQVYTLPPSRDELTKNQVSLTCLVKGFYPSDIAVEWESNGQPENNYKTTPPVLDSDGSFFLYSKLTVDKSRWQQGNVFSCSVMHEALHNHYTQKSLSLSPGKLPETGGWSHPQFEK

SEQ ID NO: 155 - protein, 236 aa, Artificial sequence
  Synthetic sequence
ELVMTQTPSSTSGAVGGTVTINCQASQSIDSNLAWFQQKPGQPPTLLIYRASNLASGVPSRFSGSRSGTEYTLTISGVQREDAATYYCLGGVGNVSYRTSFGGGTEVVVKRTVAAPSVFIFPPSDEQLKSGTASVVCLLNNFYPREAKVQWKVDNALQSGNSQESVTEQDSKDSTYSLSSTLTLSKADYEKHKVYACEVTHQGLSSPVTKSFNRGECGGGGSLPETGGWSHPQFEK

SEQ ID NO: 156 - protein, 465 aa, Artificial sequence
  Synthetic sequence
QEQLVESGGRLVTPGGSLTLSCKASGFDFSAYYMSWVRQAPGKGLEWIATIYPSSGKTYYATWVNGRFTISSDNAQNTVDLQMNSLTAADRATYFCARDSYADDGALFNIWGPGTLVTISSASTKGPSVFPLAPSSKSTSGGTAALGCLVKDYFPEPVTVSWNSGALTSGVHTFPAVLQSSGLYSLSSVVTVPSSSLGTQTYICNVNHKPSNTKVDKKVEPKSCDKTHTCPPCPAPELLGGPSVFLFPPKPKDTLMISRTPEVTCVVVDVSHEDPEVKFNWYVDGVEVHNAKTKPREEQYNSTYRVVSVLTVLHQDWLNGKEYKCKVSNKALPAPIEKTISKAKGQPREPQVYTLPPSRDELTKNQVSLTCLVKGFYPSDIAVEWESNGQPENNYKTTPPVLDSDGSFFLYSKLTVDKSRWQQGNVFSCSVMHEALHNHYTQKSLSLSPGKLPETGGWSHPQFEK

SEQ ID NO: 157 - protein, 236 aa, Artificial sequence
  Synthetic sequence
ELVLTQSPSVSAALGSPAKITCTLSSAHKTDTIDWYQQLQGEAPRYLMQVQSDGSYTKRPGVPDRFSGSSSGADRYLIIPSVQADDEADYYCGADYIGGYVFGGGTQLTVTGQPKAAPSVTLFPPSSEELQANKATLVCLISDFYPGAVTVAWKADSSPVKAGVETTTPSKQSNNKYAASSYLSLTPEQWKSHKSYSCQVTHEGSTVEKTVAPTECSGGGGSLPETGGWSHPQFEK

SEQ ID NO: 158 - protein, 450 aa, Artificial sequence
  Synthetic sequence
EVQLVESGGGLVQPGGSLRLSCAASGFNIKDTYIHWVRQAPGKGLEWVARIYPTNGYTRYADSVKGRFTISADTSKNTAYLQMNSLRAEDTAVYYCSRWGGDGFYAMDYWGQGTLVTVSSASTKGPSVFPLAPSSKSTSGGTAALGCLVKDYFPEPVTVSWNSGALTSGVHTFPAVLQSSGLYSLSSVVTVPSSSLGTQTYICNVNHKPSNTKVDKKVEPKSCDKTHTCPPCPAPELLGGPSVFLFPPKPKDTLMISRTPEVTCVVVDVSHEDPEVKFNWYVDGVEVHNAKTKPREEQYNSTYRVVSVLTVLHQDWLNGKEYKCKVSNKALPAPIEKTISKAKGQPREPQVYTLPPSRDELTKNQVSLTCLVKGFYPSDIAVEWESNGQPENNYKTTPPVLDSDGSFFLYSKLTVDKSRWQQGNVFSCSVMHEALHNHYTQKSLSLSPGK

SEQ ID NO: 159 - protein, 214 aa, Artificial sequence
  Synthetic sequence
DIQMTQSPSSLSASVGDRVTITCRASQDVNTAVAWYQQKPGKAPKLLIYSASFLYSGVPSRFSGSRSGTDFTLTISSLQPEDFATYYCQQHYTTPPTFGQGTKVEIKRTVAAPSVFIFPPSDEQLKSGTASVVCLLNNFYPREAKVQWKVDNALQSGNSQESVTEQDSKDSTYSLSSTLTLSKADYEKHKVYACEVTHQGLSSPVTKSFNRGEC

SEQ ID NO: 160 - protein, 461 aa, Artificial sequence
  Synthetic sequence
QIQLQQSGPEVVKPGASVKISCKASGYTFTDYYITWVKQKPGQGLEWIGWIYPGSGNTKYNEKFKGKATLTVDTSSSTAFMQLSSLTSEDTAVYFCANYGNYWFAYWGQGTQVTVSAASTKGPSVFPLAPSSKSTSGGTAALGCLVKDYFPEPVTVSWNSGALTSGVHTFPAVLQSSGLYSLSSVVTVPSSSLGTQTYICNVNHKPSNTKVDKKVEPKSCDKTHTCPPCPAPELLGGPSVFLFPPKPKDTLMISRTPEVTCVVVDVSHEDPEVKFNWYVDGVEVHNAKTKPREEQYNSTYRVVSVLTVLHQDWLNGKEYKCKVSNKALPAPIEKTISKAKGQPREPQVYTLPPSRDELTKNQVSLTCLVKGFYPSDIAVEWESNGQPENNYKTTPPVLDSDGSFFLYSKLTVDKSRWQQGNVFSCSVMHEALHNHYTQKSLSLSPGKLPETGGWSHPQFEK

SEQ ID NO: 161 - protein, 237 aa, Artificial sequence
  Synthetic sequence
DIVLTQSPASLAVSLGQRATISCKASQSVDFDGDSYMNWYQQKPGQPPKVLIYAASNLESGIPARFSGSGSGTDFTLNIHPVEEEDAATYYCQQSNEDPWTFGGGTKLEIKRTVAAPSVFIFPPSDEQLKSGTASVVCLLNNFYPREAKVQWKVDNALQSGNSQESVTEQDSKDSTYSLSSTLTLSKADYEKHKVYACEVTHQGLSSPVTKSFNRGECGGGGSLPETGGWSHPQFEK